European Patent Specification EP 4 034 104 B1, published August 6, 2025. Title: METHODS AND COMPOUNDS FOR RESTORING MUTANT P53 FUNCTION. Applicant: PMV PHARMACEUTICALS, INC. Application Herewith. The sequence listing filed with the application follows.

SEQUENCE LISTING (2 sequences)

SEQ ID NO: 1 - protein, 219 aa, Artificial Sequence
  Description of Artificial Sequence: Synthetic polypeptide
SSSVPSQKTYQGSYGFRLGFLHSGTAKSVTCTYSPALNKMFCQLAKTCPVQLWVDSTPPPGTRVRAMAIYKQSQHMTEVVRRCPHHERCSDSDGLAPPQHLIRVEGNLRVEYLDDRNTFRHSVVVPCEPPEVGSDCTTIHYNYMCNSSCMGGMNRRPILTIITLEDSSGNLLGRNSFEVHVCACPGRDRRTEEENLRKKGEPHHELPPGSTKRALSNNT

SEQ ID NO: 2 - DNA, 26 bp, Artificial Sequence
  Description of Artificial Sequence: Synthetic oligonucleotide
attaggcatgtctaggcatgtctagg